European Patent Application EP 4 715 046 A1, published March 25, 2026. Title: 신규한 PET 분해 효소 및 그 용도. Applicant: 주식회사 자이엔. The sequence listing filed with the application follows.

SEQUENCE LISTING (13 sequences)

SEQ ID NO: 1 - protein, 299 aa, Cryptosporangium aurantiacum
  source 1..299: note = CaPETase WT
MLSFLRSTGRPERRRASLPALLLFTAALVASGLTAAPAAQAADNPYQRGPDPTNASIEAATGPFAVGTQPIVGASGFGGGQIYYPTDTSQTYGAVVIVPGFISVWAQLNWLGPRLASQGFVVIGIETSVITDLPDPRGDQALAALDWATTRSPVASRIDRTRLAAAGWSMGGGGLRRAALQRPSLKAIVGMAPWNGERNWSAVTVPTLFFGGSSDAVASPNDHAKPFYNSITRAEKDYIELRNADHFFPTSANTTMAKYFISWLKRWVDNDTRYTQFLCPGPSTGLFAPVSASMNTCPF

SEQ ID NO: 2 - DNA, 900 bp, Cryptosporangium aurantiacum
  source 1..900: mol_type = genomic DNA; note = CaPETase WT
gtgctgtcctttctccgaagtaccggccgccccgagcgccgacgagcgtcgttaccggcgctcctgttgttcaccgctgcgctcgtcgcgagcgggctcaccgccgcccccgccgcgcaggcggccgacaacccctaccaacgcggtccggaccccacgaacgcgagtatcgaggcggcgaccggcccgttcgcggtcggcacgcagccgatcgtcggtgcctccggcttcggcggcggccagatctactacccgaccgacaccagccagacgtacggggcggtcgtgatcgtgccgggcttcatctcggtctgggcccagctcaactggctcgggccgcgcctggcgtcccagggttttgtggtcatcggcatcgagaccagcgtgatcaccgacctgcccgacccgcgcggtgaccaggcgctggccgcgctggactgggcgacgacccggagcccggtcgcgagccggatcgaccggacccggctggccgcggccggctggtcgatgggcggcggcggcctgcggcgggccgcactgcaacgcccgtcgctcaaggcgatcgtcgggatggcgccctggaacggcgagcgcaactggtccgccgtcaccgtgccgacgctgttcttcggtggttcgtccgacgccgtcgcctcgccgaacgaccacgcgaagccgttctacaacagcatcacccgagccgagaaggattacatcgaactccggaacgccgaccatttcttccccacgtcggcgaacaccacgatggcgaaatacttcatctcgtggctcaagcgttgggtggacaacgacacccgctacacccagttcctctgccccggaccgtccaccggattgttcgccccggtgagcgcgtcgatgaacacctgcccgttctga

SEQ ID NO: 3 - protein, 299 aa, synthetic construct
  source 1..299: note = CaPETaseM1
MLSFLRSTGRPERRRASLPALLLFTAALVASGLTAAPAAQAADNPYQRGPDPTNASIEAATGPFAVGTQPIVGASGFGGGQIYYPTDTSQTYGAVVIVPGFISVWAQLAWLGPRLASQGFVVIGIETSVITDLPDPRGDQALAALDWATTRSPVASRIDRTRLAAAGWSMGGGGLRRAALQRPSLKAIVGMAPWNGERNWSAVTVPTLFFGGSSDAVASPNDHAKPFYNSITRAEKDYIELRNADHFFPTSANTTMAKYFISWLKRWVDNDTRYTQFLCPGPSTGLFAPVSASMNTCPF

SEQ ID NO: 4 - protein, 299 aa, synthetic construct
  source 1..299: note = CaPETaseM2
MLSFLRSTGRPERRRASLPALLLFTAALVASGLTAAPAAQAADNPYQRGPDPTNASIEAATGPFAVGTQPIVGASGFGGGQIYYPTDTSQTYGAVVIVPGFISVWAQLNWLGPRLASQGFVVIGIETSVITDLPDPRGDQALAALDWATTRSPVRSRIDRTRLAAAGWSMGGGGLRRAALQRPSLKAIVGMAPWNGERNWSAVTVPTLFFGGSSDAVASPNDHAKPFYNSITRAEKDYIELRNADHFFPTSANTTMAKYFISWLKRWVDNDTRYTQFLCPGPSTGLFAPVSASMNTCPF

SEQ ID NO: 5 - protein, 299 aa, synthetic construct
  source 1..299: note = CaPETaseM3
MLSFLRSTGRPERRRASLPALLLFTAALVASGLTAAPAAQAADNPYQRGPDPTNASIEAATGPFAVGTQPIVGASGFGGGQIYYPTDTSQTYGAVVIVPGFISVWAQLAWLGPRLASQGFVVIGIETSVITDLPDPRGDQALAALDWATTRSPVRSRIDRTRLAAAGWSMGGGGLRRAALQRPSLKAIVGMAPWNGERNWSAVTVPTLFFGGSSDAVASPNDHAKPFYNSITRAEKDYIELRNADHFFPTSANTTMAKYFISWLKRWVDNDTRYTQFLCPGPSTGLFAPVSASMNTCPF

SEQ ID NO: 6 - DNA, 33 bp, synthetic construct
  source 1..33: mol_type = other DNA
tatatcatatggcggccgacaacccctaccaac

SEQ ID NO: 7 - DNA, 33 bp, synthetic construct
  source 1..33: mol_type = other DNA
tatatctcgaggaacgggcaggtgttcatcgac

SEQ ID NO: 8 - DNA, 34 bp, synthetic construct
  source 1..34: mol_type = other DNA
tatacatatgcgcggtccgaatccgacagccgcc

SEQ ID NO: 9 - DNA, 34 bp, synthetic construct
  source 1..34: mol_type = other DNA
gcgcctcgaggctgcaattcgctgtacgaaaatc

SEQ ID NO: 10 - DNA, 30 bp, synthetic construct
  source 1..30: mol_type = other DNA
gcgccatatggccaacccctacgaacgtgg

SEQ ID NO: 11 - DNA, 27 bp, synthetic construct
  source 1..27: mol_type = other DNA
gcgcctcgaggaatgggcaggtcgagc

SEQ ID NO: 12 - DNA, 34 bp, synthetic construct
  source 1..34: mol_type = other DNA
tatatcatatgcaatccaacccgtaccagcgcgg

SEQ ID NO: 13 - DNA, 33 bp, synthetic construct
  source 1..33: mol_type = other DNA
tatatctcgagctggcagtggcggttgttcgtc